European Patent Application EP 4 230 732 A1, published August 23, 2023. Title: RECOMBINANT CHO CELL, CONSTRUCTION METHOD THEREFOR, AND DETECTION SYSTEM AND METHODD USING SAME. Applicant: CHENGDU UNOVEL BIOPHARMA CO., LTD. The sequence listing filed with the application follows.

SEQUENCE LISTING (17 sequences)

SEQ ID NO: 1 - protein, 241 aa, Homo sapiens
MSMLFYTLITAFLIGIQAEPHSESNVPAGHTIPQAHWTKLQHSLDTALRRARSAPAAAIAARVAGQTRNITVDPRLFKKRRLRSPRVLFSTQPPREAADTQDLDFEVGGAAPFNRTHRSKRSSSHPIFHRGEFSVCDSVSVWVGDKTTATDIKGKEVMVLGEVNINNSVFKQYFFETKCRDPNPVDSGCRGIDSKHWNSYCTTTHTFVKALTMDGKQAAWRFIRIDTACVCVLSRKAVRRA

SEQ ID NO: 2 - protein, 120 aa, Homo sapiens
SSSHPIFHRGEFSVCDSVSVWVGDKTTATDIKGKEVMVLGEVNINNSVFKQYFFETKCRDPNPVDSGCRGIDSKHWNSYCTTTHTFVKALTMDGKQAAWRFIRIDTACVCVLSRKAVRRA

SEQ ID NO: 3 - protein, 118 aa, Homo sapiens
SSSHPIFHRGEFSVCDSVSVWVGDKTTATDIKGKEVMVLGEVNINNSVFKQYFFETKCRDPNPVDSGCRGIDSKHWNSYCTTTHTFVKALTMDGKQAAWRFIRIDTACVCVLSRKAVR

SEQ ID NO: 4 - DNA, 723 bp, Homo sapiens
atgagcatgctgttctataccctgatcaccgcctttctgatcggcatccaggccgagcctcacagcgagtctaatgtgcctgccggccacacaatccctcaggctcactggacaaagctgcagcacagcctggatacagctctgcggagagccagatctgctcctgccgctgctattgccgctagagtggctggccagaccagaaacatcaccgtggatccccggctgttcaagaagcggagactgagaagccccagagtgctgttcagcacccagcctccaagagaggccgccgatacacaggacctggattttgaagttggcggcgctgcccctttcaacagaacccacagaagcaagcggagcagctctcaccccatcttccacagaggcgagttcagcgtgtgcgactccgtgtctgtgtgggtcggagataagaccaccgccaccgacatcaagggcaaagaagtgatggtcctgggcgaagtgaacatcaacaacagcgtgttcaagcagtacttcttcgagacaaagtgcagggaccccaatcctgtggacagcggctgtagaggcatcgacagcaagcactggaactcctactgcaccaccacacacaccttcgtgaaggccctgaccatggatggaaaacaggccgcctggcggttcatcagaatcgataccgcttgcgtgtgcgtgctgagcagaaaagccgttagaagggcc

SEQ ID NO: 5 - DNA, 360 bp, Homo sapiens
agcagctctcaccccatcttccacagaggcgagttcagcgtgtgcgactccgtgtctgtgtgggtcggagataagaccaccgccaccgacatcaagggcaaagaagtgatggtcctgggcgaagtgaacatcaacaacagcgtgttcaagcagtacttcttcgagacaaagtgcagggaccccaatcctgtggacagcggctgtagaggcatcgacagcaagcactggaactcctactgcaccaccacacacaccttcgtgaaggccctgaccatggatggaaaacaggccgcctggcggttcatcagaatcgataccgcttgcgtgtgcgtgctgagcagaaaagccgttagaagggcc

SEQ ID NO: 6 - DNA, 354 bp, Homo sapiens
agcagctctcaccccatcttccacagaggcgagttcagcgtgtgcgactccgtgtctgtgtgggtcggagataagaccaccgccaccgacatcaagggcaaagaagtgatggtcctgggcgaagtgaacatcaacaacagcgtgttcaagcagtacttcttcgagacaaagtgcagggaccccaatcctgtggacagcggctgtagaggcatcgacagcaagcactggaactcctactgcaccaccacacacaccttcgtgaaggccctgaccatggatggaaaacaggccgcctggcggttcatcagaatcgataccgcttgcgtgtgcgtgctgagcagaaaagccgttaga

SEQ ID NO: 7 - protein, 45 aa, Artificial Sequence
  Amino acid sequence of CD8 hinge region
TTTPAPRPPTPAPTIASQPLSLRPEACRPAAGGAVHTRGLDFACD

SEQ ID NO: 8 - protein, 12 aa, Homo sapiens
EPKSCDKTHTCP

SEQ ID NO: 9 - DNA, 135 bp, Artificial Sequence
  Nucleic acid sequence of CD8 hinge region
accactaccccagcaccgaggccacccaccccggctcctaccatcgcctcccagcctctgtccctgcgtccggaggcatgtagacccgcagctggtggggccgtgcatacccgtggtcttgacttcgcctgcgat

SEQ ID NO: 10 - protein, 24 aa, Artificial Sequence
  Amino acid sequence of CD8 transmembrane region
IYIWAPLAGTCGVLLLSLVITLYC

SEQ ID NO: 11 - protein, 21 aa, Artificial Sequence
  Amino acid sequence of the transmembrane region of PGFRA
AAVLVLLVIVIISLIVLVVIW

SEQ ID NO: 12 - protein, 21 aa, Artificial Sequence
  Amino acid sequence of CD80 transmembrane region
LLPSWAITLISVNGIFVICCL

SEQ ID NO: 13 - DNA, 72 bp, Artificial Sequence
  Nucleic acid sequence of CD8 transmembrane region
atctacatttgggcccctctggctggtacttgcggggtcctgctgctttcactcgtgatcactctttactgt

SEQ ID NO: 14 - protein, 447 aa, Unknown
  The heavy chain sequence of Tanezumab
QVQLQESGPGLVKPSETLSLTCTVSGFSLIGYDLNWIRQPPGKGLEWIGIIWGDGTTDYNSAVKSRVTISKDTSKNQFSLKLSSVTAADTAVYYCARGGYWYATSYYFDYWGQGTLVTVSSASTKGPSVFPLAPCSRSTSESTAALGCLVKDYFPEPVTVSWNSGALTSGVHTFPAVLQSSGLYSLSSVVTVPSSNFGTQTYTCNVDHKPSNTKVDKTVERKCCVECPPCPAPPVAGPSVFLFPPKPKDTLMISRTPEVTCVVVDVSHEDPEVQFNWYVDGVEVHNAKTKPREEQFNSTFRVVSVLTVVHQDWLNGKEYKCKVSNKGLPSSIEKTISKTKGQPREPQVYTLPPSREEMTKNQVSLTCLVKGFYPSDIAVEWESNGQPENNYKTTPPMLDSDGSFFLYSKLTVDKSRWQQGNVFSCSVMHEALHNHYTQKSLSLSPGK

SEQ ID NO: 15 - protein, 214 aa, Unknown
  The light chain sequence of Tanezumab
DIQMTQSPSSLSASVGDRVTITCRASQSISNNLNWYQQKPGKAPKLLIYYTSRFHSGVPSRFSGSGSGTDFTFTISSLQPEDIATYYCQQEHTLPYTFGQGTKLEIKRTVAAPSVFIFPPSDEQLKSGTASVVCLLNNFYPREAKVQWKVDNALQSGNSQESVTEQDSKDSTYSLSSTLTLSKADYEKHKVYACEVTHQGLSSPVTKSFNRGEC

SEQ ID NO: 16 - protein, 330 aa, Homo sapiens [sequence omitted]

SEQ ID NO: 17 - DNA, 993 bp, Homo sapiens
gcctctacaaagggcccctccgtttttccactggctcccagcagcaagtctacctctggtggaacagccgctctgggctgcctggtcaaggattactttcccgagccagtgaccgtgtcctggaactctggcgctctgacatctggcgtgcacacatttccagccgtgctgcagtctagcggcctgtactctctgagcagcgtggtcacagtgcctagctctagcctgggcacccagacctacatctgcaatgtgaaccacaagcctagcaacaccaaggtggacaagaaggtggaacccaagagctgcgacaagacccacacctgtcctccatgtcctgctccagaactgctcggcggaccttccgtgtttctgttccctccaaagcctaaggacaccctgatgatcagcagaacccctgaagtgacctgcgtggtggtggatgtgtcccacgaggaccccgaagtgaagttcaattggtacgtggacggcgtggaagtgcacaacgccaagaccaagcctagagaggaacagtacaacagcacctacagagtggtgtccgtgctgacagtgctgcatcaggactggctgaacggcaaagagtacaagtgcaaggtgtccaacaaggccctgcctgctcctatcgagaaaaccatcagcaaggccaagggccagcctagggaaccccaggtttacacactgcctccaagcagggacgagctgaccaagaatcaggtgtccctgacctgcctcgtgaagggcttctacccttccgatatcgccgtggaatgggagagcaatggccagcctgagaacaactacaagacaacccctcctgtgctggacagcgacggctcattcttcctgtacagcaagctgaccgtggacaagtccagatggcagcagggcaacgtgttcagctgctccgtgatgcacgaggccctgcacaaccactacacccagaagtccctgagcctgtctcctggcaaataa